European Patent Application EP 4 159 873 A1, published April 5, 2023. Title: A method of analyzing a population of cells and method of analyzing genes included in a population of cells. Applicant: RIKEN. The sequence listing filed with the application follows.

SEQUENCE LISTING (34 sequences)

SEQ ID NO: 1 - DNA, 17 bp, Artificial Sequence
  341F
  misc_feature (9)..(9): n is a, c, g, or t
cctacgggnggcwgcag

SEQ ID NO: 2 - DNA, 21 bp, Artificial Sequence
  805R
gactachvgggtatctaatcc

SEQ ID NO: 3 - DNA, 74 bp, Artificial Sequence
  P7-R2P-341F
  misc_feature (66)..(66): n is a, c, g, or t
caagcagaagacggcatacgagatgtgactggagttccttggcacccgagaattccacctacgggnggcwgcag

SEQ ID NO: 4 - DNA, 45 bp, Artificial Sequence
  Biotin-link-805R
  modified_base (1)..(1): modified with biotin
  modified_base (28)..(28): modified with biotin
gctcctgcgttcggatcgtagtcggactachvgggtatctaatcc

SEQ ID NO: 5 - DNA, 44 bp, Artificial Sequence
  Biotin-Link-barcode-F
  modified_base (1)..(1): modified with biotin
  modified_base (31)..(31): modified with biotin
cgactacgatccgaacgcaggagctcagcctcgacagtccagtg

SEQ ID NO: 6 - DNA, 70 bp, Artificial Sequence
  P5-index-R1P-barcode-R
  misc_feature (30)..(37): n is a, c, g, or t
aatgatacggcgaccaccgagatctacacnnnnnnnnacactctttccctacacgacgctcttccgatct

SEQ ID NO: 7 - DNA, 44 bp, Artificial Sequence; identical to SEQ ID NO: 5
  NoBiotin-Link-barcode

SEQ ID NO: 8 - DNA, 20 bp, Artificial Sequence
  F1-Fw
agrgtttgatymtggctcag

SEQ ID NO: 9 - DNA, 17 bp, Artificial Sequence
  F1-Rv
ctggcacgdagttagcc

SEQ ID NO: 10 - DNA, 77 bp, Artificial Sequence
  F1-full-Fw
caagcagaagacggcatacgagatgtgactggagttccttggcacccgagaattccaagrgtttgatymtggctcag

SEQ ID NO: 11 - DNA, 46 bp, Artificial Sequence
  F3-full-Rv
gctcctgcgttcggatcgtagtcgtacggytaccttgttacgactt

SEQ ID NO: 12 - DNA, 18 bp, Artificial Sequence
  T7-Promoter
taatacgactcactatag

SEQ ID NO: 13 - DNA, 18 bp, Artificial Sequence
  SP6-Promoter
atttaggtgacactatag

SEQ ID NO: 14 - DNA, 23 bp, Artificial Sequence
  F2-Rv
cttgtgcgggcccccgtcaattc

SEQ ID NO: 15 - DNA, 83 bp, Artificial Sequence
  Barcode-1
  misc_feature (23)..(26): n is a, c, g, or t
  misc_feature (28)..(31): n is a, c, g, or t
  misc_feature (33)..(36): n is a, c, g, or t
  misc_feature (38)..(41): n is a, c, g, or t
  misc_feature (43)..(50): n is a, c, g, or t
tcagcctcgacagtccagtgacnnnntnnnngnnnnannnncnnnnnnnnagatcggaagagcgtcgtgtagggaaagagtgt

SEQ ID NO: 16 - DNA, 83 bp, Artificial Sequence
  Barcode-2
  misc_feature (23)..(26): n is a, c, g, or t
  misc_feature (28)..(31): n is a, c, g, or t
  misc_feature (33)..(36): n is a, c, g, or t
  misc_feature (38)..(41): n is a, c, g, or t
  misc_feature (43)..(50): n is a, c, g, or t
tcagcctcgacagtccagtgtgnnnnannnncnnnntnnnngnnnnnnnnagatcggaagagcgtcgtgtagggaaagagtgt

SEQ ID NO: 17 - DNA, 83 bp, Artificial Sequence
  Barcode-3
  misc_feature (23)..(26): n is a, c, g, or t
  misc_feature (28)..(31): n is a, c, g, or t
  misc_feature (33)..(36): n is a, c, g, or t
  misc_feature (38)..(41): n is a, c, g, or t
  misc_feature (43)..(50): n is a, c, g, or t
tcagcctcgacagtccagtggannnncnnnnannnngnnnntnnnnnnnnagatcggaagagcgtcgtgtagggaaagagtgt

SEQ ID NO: 18 - DNA, 83 bp, Artificial Sequence
  Barcode-4
  misc_feature (23)..(26): n is a, c, g, or t
  misc_feature (28)..(31): n is a, c, g, or t
  misc_feature (33)..(36): n is a, c, g, or t
  misc_feature (38)..(41): n is a, c, g, or t
  misc_feature (43)..(50): n is a, c, g, or t
tcagcctcgacagtccagtgctnnnngnnnntnnnncnnnnannnnnnnnagatcggaagagcgtcgtgtagggaaagagtgt

SEQ ID NO: 19 - DNA, 21 bp, Artificial Sequence
  P1_qPCR_Fw
aatgatacggcgcaccaccga

SEQ ID NO: 20 - DNA, 21 bp, Artificial Sequence
  P2_qPCR_Rv
caagcagaagacggcatacga

SEQ ID NO: 21 - DNA, 200 bp, Artificial Sequence
  StdTarget1
  misc_feature (27)..(200): n is a, c, g, or t
gagttccttggcacccgagaattccannnnnnnnnnnnnnnnnnnnnnnnnnnnnnnnnnnnnnnnnnnnnnnnnnnnnnnnnnnnnnnnnnnnnnnnnnnnnnnnnnnnnnnnnnnnnnnnnnnnnnnnnnnnnnnnnnnnnnnnnnnnnnnnnnnnnnnnnnnnnnnnnnnnnnnnnnnnnnnnnnnnnnnnnnnnnn

SEQ ID NO: 22 - DNA, 200 bp, Artificial Sequence
  StdTarget2
  modified_base (1)..(1): modified with phosphate
  misc_feature (1)..(176): n is a, c, g, or t
nnnnnnnnnnnnnnnnnnnnnnnnnnnnnnnnnnnnnnnnnnnnnnnnnnnnnnnnnnnnnnnnnnnnnnnnnnnnnnnnnnnnnnnnnnnnnnnnnnnnnnnnnnnnnnnnnnnnnnnnnnnnnnnnnnnnnnnnnnnnnnnnnnnnnnnnnnnnnnnnnnnnnnnnnnnnnnnncgactacgatccgaacgcaggagc

SEQ ID NO: 23 - DNA, 99 bp, Artificial Sequence
  RandomBar_std1
  misc_feature (27)..(34): n is a, c, g, or t
  misc_feature (36)..(39): n is a, c, g, or t
  misc_feature (41)..(44): n is a, c, g, or t
  misc_feature (46)..(49): n is a, c, g, or t
  misc_feature (51)..(54): n is a, c, g, or t
ttccctacacgacgctcttccgatctnnnnnnnncnnnntnnnnannnngnnnnctcactggactgtcgaggctgagctcctgcgttcggatcgtagtc

SEQ ID NO: 24 - DNA, 99 bp, Artificial Sequence
  RandomBar_std2
  misc_feature (27)..(34): n is a, c, g, or t
  misc_feature (36)..(39): n is a, c, g, or t
  misc_feature (41)..(44): n is a, c, g, or t
  misc_feature (46)..(49): n is a, c, g, or t
  misc_feature (51)..(54): n is a, c, g, or t
ttccctacacgacgctcttccgatctnnnnnnnngnnnnannnntnnnnannnntgcactggactgtcgaggctgagctcctgcgttcggatcgtagtc

SEQ ID NO: 25 - DNA, 99 bp, Artificial Sequence
  RandomBar_std3
  misc_feature (27)..(34): n is a, c, g, or t
  misc_feature (36)..(39): n is a, c, g, or t
  misc_feature (41)..(44): n is a, c, g, or t
  misc_feature (46)..(49): n is a, c, g, or t
  misc_feature (51)..(54): n is a, c, g, or t
ttccctacacgacgctcttccgatctnnnnnnnntnnnncnnnngnnnncnnnngacactggactgtcgaggctgagctcctgcgttcggatcgtagtc

SEQ ID NO: 26 - DNA, 99 bp, Artificial Sequence
  RandomBar_std4
  misc_feature (27)..(34): n is a, c, g, or t
  misc_feature (36)..(39): n is a, c, g, or t
  misc_feature (41)..(44): n is a, c, g, or t
  misc_feature (46)..(49): n is a, c, g, or t
  misc_feature (51)..(54): n is a, c, g, or t
ttccctacacgacgctcttccgatctnnnnnnnnannnngnnnncnnnntnnnnaccactggactgtcgaggctgagctcctgcgttcggatcgtagtc

SEQ ID NO: 27 - DNA, 70 bp, Artificial Sequence
  Index_NSE501
aatgatacggcgaccaccgagatctacactagatcgcacactctttccctacacgacgctcttccgatct

SEQ ID NO: 28 - DNA, 70 bp, Artificial Sequence
  Index_NSE502
aatgatacggcgaccaccgagatctacacctctctatacactctttccctacacgacgctcttccgatct

SEQ ID NO: 29 - DNA, 70 bp, Artificial Sequence
  Index_NSE505
aatgatacggcgaccaccgagatctacacgtaaggagacactctttccctacacgacgctcttccgatct

SEQ ID NO: 30 - DNA, 70 bp, Artificial Sequence
  Index_NSE506
aatgatacggcgaccaccgagatctacacactgcataacactctttccctacacgacgctcttccgatct

SEQ ID NO: 31 - DNA, 57 bp, Artificial Sequence
  std_R2
caagcagaagacggcatacgagatgtgactggagttccttggcacccgagaattcca

SEQ ID NO: 32 - DNA, 28 bp, Artificial Sequence
  I1_primer
ctgagctcctgcgttcggatcgtagtcg

SEQ ID NO: 33 - DNA, 50 bp, Artificial Sequence
  CONV- 341F
  misc_feature (42)..(42): n is a, c, g, or t
tcgtcggcagcgtcagatgtgtataagagacagcctacgggnggcwgcag

SEQ ID NO: 34 - DNA, 55 bp, Artificial Sequence
  CONV- 806R
gtctcgtgggctcggagatgtgtataagagacaggactachvgggtatctaatcc